European Patent Application EP 4 574 963 A1, published June 25, 2025. Title: LACTOBACILLUS RHAMNOSUS AND COMPOSITION FOR INHIBITING H.PYLORI. Applicant: Bloomage Biotechnology Corporation Limited. The sequence listing filed with the application follows.

SEQUENCE LISTING (1 sequence)

SEQ ID NO: 1 - RNA, 1448 nt, synthetic construct
  source 1..1448: mol_type = other RNA
cttagacggctcgctccctaaagggttacgccaccggcttcgggtgttacaaactctcatggtgtgacgggcggtgtgtacaaggcccgggaacgtattcaccgcggcgtgctgatccgcgattactagcgattccgacttcgtgtaggcgagttgcagcctacagtccgaactgagaatggctttaagagattagcttgacctcgcggtctcgcaactcgttgtaccatccattgtagcacgtgtgtagcccaggtcataaggggcatgatgatttgacgtcatccccaccttcctccggtttgtcaccggcagtcttactagagtgcccaactaaatgctggcaactagtcataagggttgcgctcgttgcgggacttaacccaacatctcacgacacgagctgacgacaaccatgcaccacctgtcattttgcccccgaaggggaaacctgatctctcaggtgatcaaaagatgtcaagacctggtaaggttcttcgcgttgcttcgaattaaaccacatgctccaccgcttgtgcgggcccccgtcaattcctttgagtttcaaccttgcggtcgtactccccaggcggaatgcttaatgcgttagctgcggcactgaagggcggaaaccctccaacacctagcattcatcgtttacggcatggactaccagggtatctaatcctgttcgctacccatgctttcgagcctcagcgtcagttacagaccagacagccgccttcgccactggtgttcttccatatatctacgcatttcaccgctacacatggagttccactgtcctcttctgcactcaagtttcccagtttccgatgcacttcctcggttaagccgagggctttcacatcagacttaaaaaaccgcctgcgctcgctttacgcccaataaatccggataacgcttgccacctacgtattaccgcggctgctggcacgtagttagccgtggctttctggttggataccgtcacgccgacaacagttactctgccgaccattcttctccaacaacagagttttacgacccgaaagccttcttcactcacgcggcgttgctccatcagacttgcgtccattgtggaagattccctactgctgcctcccgtaggagtttgggccgtgtctcagtcccaatgtggccgatcaacctctcagttcggctacgtatcattgccttggtgagccgttacctcaccaactagctaatacgccgcgggtccatccaaaagcgatagcttacgccatctttcagccaagaaccatgcggttcttggatttatgcggtattagcatctgtttccaaatgttatcccccacttaagggcaggttacccacgtgttactcacccgtccgccactcgttcaaaattaaatcaagatgcaagcacctttcaataatcagaactcgttcgactgcatgtatag